European Patent Specification EP 3 326 453 B9, published October 4, 2023. Title: ALS inhibitor herbicide tolerance Beta vulgaris mutants. Applicant: Bayer Intellectual Property GmbH and KWS SAAT SE. The sequence listing filed with the application follows.

SEQUENCE LISTING (6 sequences)

SEQ ID NO: 1 - DNA, 1998 bp, Beta vulgaris
atggcggctaccttcacaaacccaacattttccccttcctcaactccattaaccaaaaccctaaaatcccaatcttccatctcttcaaccctccccttttccacccctcccaaaaccccaactccactctttcaccgtcccctccaaatctcatcctcccaatcccacaaatcatccgccattaaaacacaaactcaagcaccttcttctccagctattgaagattcatctttcgtttctcgatttggccctgatgaacccagaaaagggtccgatgtcctcgttgaagctcttgagcgtgaaggtgttaccaatgtgtttgcttaccctggtggtgcatctatggaaatccaccaagctctcacacgctctaaaaccatccgcaatgtcctccctcgccatgaacaaggcggggttttcgccgccgagggatatgctagagctactggaaaggttggtgtctgcattgcgacttctggtcctggtgctaccaacctcgtatcaggtcttgctgacgctctccttgattctgtccctcttgttgccatcactggccaagttccacgccgtatgattggcactgatgcttttcaggagactccaattgttgaggtgacaaggtctattactaagcataattatttagttttggatgtagaggatattcctagaattgttaaggaagccttttttttagctaattctggtaggcctggacctgttttgattgatcttcctaaagatattcagcagcaattggttgttcctgattgggataggccttttaagttgggtgggtatatgtctaggctgccaaagtccaagttttcgacgaatgaggttggacttcttgagcagattgtgaggttgatgagtgagtcgaagaagcctgtcttgtatgtgggaggtgggtgtttgaattctagtgaggagttgaggagatttgttgagttgacagggattccggtggctagtactttgatggggttggggtcttacccttgtaatgatgaactgtctcttcatatgttggggatgcacgggactgtttatgccaattatgcggtggataaggcggatttgttgcttgctttcggggttaggtttgatgatcgtgtgaccgggaagctcgaggcgtttgctagccgtgctaagattgtgcatattgatattgactctgctgagattgggaagaacaagcagccccatgtgtccatttgtgctgatgttaaattggcattgcggggtatgaataagattctggagtctagaatagggaagctgaatttggatttctccaagtggagagaagaattaggtgagcagaagaaggaattcccactgagttttaagacatttggggatgcaattcctccacaatatgccattcaggtgcttgatgagttgaccaatggtaatgctattataagtactggtgttgggcagcaccaaatgtgggctgcgcagcattacaagtacagaaaccctcgccaatggctgacctctggtgggttgggggctatggggtttgggctaccagccgccattggagctgcagttgctcgaccagatgcagtggttgtcgatattgatggggatggcagttttattatgaatgttcaagagttggctacaattagggtggaaaatctcccagttaagataatgctgctaaacaatcaacatttaggtatggttgtccaatgggaagataggttctataaagctaaccgggcacatacataccttggaaacccttccaaatctgctgatatcttccctgatatgctcaaattcgctgaggcatgtgatattccttctgcccgtgttagcaacgtggctgatttgagggccgccattcaaacaatgttggatactccagggccgtacctgctcgatgtgattgtaccgcatcaagagcatgtgttgcctatgattccaagtggtgccggtttcaaggataccattacagagggtgatggaagaacctcttattga

SEQ ID NO: 2 - protein, 665 aa, Beta vulgaris
MAATFTNPTFSPSSTPLTKTLKSQSSISSTLPFSTPPKTPTPLFHRPLQISSSQSHKSSAIKTQTQAPSSPAIEDSSFVSRFGPDEPRKGSDVLVEALEREGVTNVFAYPGGASMEIHQALTRSKTIRNVLPRHEQGGVFAAEGYARATGKVGVCIATSGPGATNLVSGLADALLDSVPLVAITGQVPRRMIGTDAFQETPIVEVTRSITKHNYLVLDVEDIPRIVKEAFFLANSGRPGPVLIDLPKDIQQQLVVPDWDRPFKLGGYMSRLPKSKFSTNEVGLLEQIVRLMSESKKPVLYVGGGCLNSSEELRRFVELTGIPVASTLMGLGSYPCNDELSLHMLGMHGTVYANYAVDKADLLLAFGVRFDDRVTGKLEAFASRAKIVHIDIDSAEIGKNKQPHVSICADVKLALRGMNKILESRIGKLNLDFSKWREELGEQKKEFPLSFKTFGDAIPPQYAIQVLDELTNGNAIISTGVGQHQMWAAQHYKYRNPRQWLTSGGLGAMGFGLPAAIGAAVARPDAVVVDIDGDGSFIMNVQELATIRVENLPVKIMLLNNQHLGMVVQWEDRFYKANRAHTYLGNPSKSADIFPDMLKFAEACDIPSARVSNVADLRAAIQTMLDTPGPYLLDVIVPHQEHVLPMIPSGAGFKDTITEGDGRTSY

SEQ ID NO: 3 - DNA, 1998 bp, Beta vulgaris
  mutation (1706)..(1706): Substitution of a Guanosine by a Thymidine
atggcggctaccttcacaaacccaacattttccccttcctcaactccattaaccaaaaccctaaaatcccaatcttccatctcttcaaccctccccttttccacccctcccaaaaccccaactccactctttcaccgtcccctccaaatctcatcctcccaatcccacaaatcatccgccattaaaacacaaactcaagcaccttcttctccagctattgaagattcatctttcgtttctcgatttggccctgatgaacccagaaaagggtccgatgtcctcgttgaagctcttgagcgtgaaggtgttaccaatgtgtttgcttaccctggtggtgcatctatggaaatccaccaagctctcacacgctctaaaaccatccgcaatgtcctccctcgccatgaacaaggcggggttttcgccgccgagggatatgctagagctactggaaaggttggtgtctgcattgcgacttctggtcctggtgctaccaacctcgtatcaggtcttgctgacgctctccttgattctgtccctcttgttgccatcactggccaagttccacgccgtatgattggcactgatgcttttcaggagactccaattgttgaggtgacaaggtctattactaagcataattatttagttttggatgtagaggatattcctagaattgttaaggaagccttttttttagctaattctggtaggcctggacctgttttgattgatcttcctaaagatattcagcagcaattggttgttcctgattgggataggccttttaagttgggtgggtatatgtctaggctgccaaagtccaagttttcgacgaatgaggttggacttcttgagcagattgtgaggttgatgagtgagtcgaagaagcctgtcttgtatgtgggaggtgggtgtttgaattctagtgaggagttgaggagatttgttgagttgacagggattccggtggctagtactttgatggggttggggtcttacccttgtaatgatgaactgtctcttcatatgttggggatgcacgggactgtttatgccaattatgcggtggataaggcggatttgttgcttgctttcggggttaggtttgatgatcgtgtgaccgggaagctcgaggcgtttgctagccgtgctaagattgtgcatattgatattgactctgctgagattgggaagaacaagcagccccatgtgtccatttgtgctgatgttaaattggcattgcggggtatgaataagattctggagtctagaatagggaagctgaatttggatttctccaagtggagagaagaattaggtgagcagaagaaggaattcccactgagttttaagacatttggggatgcaattcctccacaatatgccattcaggtgcttgatgagttgaccaatggtaatgctattataagtactggtgttgggcagcaccaaatgtgggctgcgcagcattacaagtacagaaaccctcgccaatggctgacctctggtgggttgggggctatggggtttgggctaccagccgccattggagctgcagttgctcgaccagatgcagtggttgtcgatattgatggggatggcagttttattatgaatgttcaagagttggctacaattagggtggaaaatctcccagttaagataatgctgctaaacaatcaacatttaggtatggttgtccaattggaagataggttctataaagctaaccgggcacatacataccttggaaacccttccaaatctgctgatatcttccctgatatgctcaaattcgctgaggcatgtgatattccttctgcccgtgttagcaacgtggctgatttgagggccgccattcaaacaatgttggatactccagggccgtacctgctcgatgtgattgtaccgcatcaagagcatgtgttgcctatgattccaagtggtgccggtttcaaggataccattacagagggtgatggaagaacctcttattga

SEQ ID NO: 4 - protein, 665 aa, Beta vulgaris
  MISC_FEATURE (569)..(569): Substitution of a Tryptophan by a Leucine
MAATFTNPTFSPSSTPLTKTLKSQSSISSTLPFSTPPKTPTPLFHRPLQISSSQSHKSSAIKTQTQAPSSPAIEDSSFVSRFGPDEPRKGSDVLVEALEREGVTNVFAYPGGASMEIHQALTRSKTIRNVLPRHEQGGVFAAEGYARATGKVGVCIATSGPGATNLVSGLADALLDSVPLVAITGQVPRRMIGTDAFQETPIVEVTRSITKHNYLVLDVEDIPRIVKEAFFLANSGRPGPVLIDLPKDIQQQLVVPDWDRPFKLGGYMSRLPKSKFSTNEVGLLEQIVRLMSESKKPVLYVGGGCLNSSEELRRFVELTGIPVASTLMGLGSYPCNDELSLHMLGMHGTVYANYAVDKADLLLAFGVRFDDRVTGKLEAFASRAKIVHIDIDSAEIGKNKQPHVSICADVKLALRGMNKILESRIGKLNLDFSKWREELGEQKKEFPLSFKTFGDAIPPQYAIQVLDELTNGNAIISTGVGQHQMWAAQHYKYRNPRQWLTSGGLGAMGFGLPAAIGAAVARPDAVVVDIDGDGSFIMNVQELATIRVENLPVKIMLLNNQHLGMVVQLEDRFYKANRAHTYLGNPSKSADIFPDMLKFAEACDIPSARVSNVADLRAAIQTMLDTPGPYLLDVIVPHQEHVLPMIPSGAGFKDTITEGDGRTSY

SEQ ID NO: 5 - DNA, 2013 bp, Arabidopsis thaliana
atggcggcggcaacaacaacaacaacaacatcttcttcgatctccttctccaccaaaccatctccttcctcctccaaatcaccattaccaatctccagattctccctcccattctccctaaaccccaacaaatcatcctcctcctcccgccgccgcggtatcaaatccagctctccctcctccatctccgccgtgctcaacacaaccaccaatgtcacaaccactccctctccaaccaaacctaccaaacccgaaacattcatctcccgattcgctccagatcaaccccgcaaaggcgctgatatcctcgtcgaagctttagaacgtcaaggcgtagaaaccgtattcgcttaccctggaggtgcatcaatggagattcaccaagccttaacccgctcttcctcaatccgtaacgtccttcctcgtcacgaacaaggaggtgtattcgcagcagaaggatacgctcgatcctcaggtaaaccaggtatctgtatagccacttcaggtcccggagctacaaatctcgttagcggattagccgatgcgttgttagatagtgttcctcttgtagcaatcacaggacaagtccctcgtcgtatgattggtacagatgcgtttcaagagactccgattgttgaggtaacgcgttcgattacgaagcataactatcttgtgatggatgttgaagatatccctaggattattgaggaagctttctttttagctacttctggtagacctggacctgttttggttgatgttcctaaagatattcaacaacagcttgcgattcctaattgggaacaggctatgagattacctggttatatgtctaggatgcctaaacctccggaagattctcatttggagcagattgttaggttgatttctgagtctaagaagcctgtgttgtatgttggtggtggttgtttgaattctagcgatgaattgggtaggtttgttgagcttacggggatccctgttgcgagtacgttgatggggctgggatcttatccttgtgatgatgagttgtcgttacatatgcttggaatgcatgggacggtgtatgcgaattacgctgtggagcatagtgatttgttgttggcgtttggggtgaggtttgatgatcgcgtcacgggtaagcttgaggcttttgctagtagggctaagattgttcatattgatattgactctgctgagattgggaagaataagactcctcatgtgtctgtgtgtggtgatgtcaagctggctttgcaagggatgaataaggttcttgagaaccgagctgaggagcttaagcttgattttggagtttggaggaatgagttgaacgtacagaaacagaagtttccgttgagctttaagacgtttggggaagctattcctccacagtatgcgattaaggtccttgatgagttgactgatggaaaagccataataagtactggtgtcgggcaacatcaaatgtgggcggcgcagttctacaattacaagaagccaaggcagtggctatcatcaggaggccttggagctatgggttttggacttcctgctgccattggagcgtctgttgctaaccctgatgcaatagttgtggatattgacggagatggaagctttataatgaatgtgcaagagctggccacaatccgtgtagagcaacttccagtgaagatactcttattaaacaaccagcatcttggcatggttatgcaatgggaagatcggttctacaaggctaaccgagctcacacatttctcggggatccggctcaggaggacgagatattcccgaacatgttgctgtttgcagcagcttgcgggattccagcggcgagggtgacaaagaaagcagatctccgagaagctattcagacaatgctggatacaccaggaccttacctgttggatgtgatttgtccgcaccaagaacatgtgttgccgatgatcccgagtggtggcactttcaacgatgtcataacggaaggagatggccggattaaatactga

SEQ ID NO: 6 - protein, 670 aa, Arabidopsis thaliana
MAAATTTTTTSSSISFSTKPSPSSSKSPLPISRFSLPFSLNPNKSSSSSRRRGIKSSSPSSISAVLNTTTNVTTTPSPTKPTKPETFISRFAPDQPRKGADILVEALERQGVETVFAYPGGASMEIHQALTRSSSIRNVLPRHEQGGVFAAEGYARSSGKPGICIATSGPGATNLVSGLADALLDSVPLVAITGQVPRRMIGTDAFQETPIVEVTRSITKHNYLVMDVEDIPRIIEEAFFLATSGRPGPVLVDVPKDIQQQLAIPNWEQAMRLPGYMSRMPKPPEDSHLEQIVRLISESKKPVLYVGGGCLNSSDELGRFVELTGIPVASTLMGLGSYPCDDELSLHMLGMHGTVYANYAVEHSDLLLAFGVRFDDRVTGKLEAFASRAKIVHIDIDSAEIGKNKTPHVSVCGDVKLALQGMNKVLENRAEELKLDFGVWRNELNVQKQKFPLSFKTFGEAIPPQYAIKVLDELTDGKAIISTGVGQHQMWAAQFYNYKKPRQWLSSGGLGAMGFGLPAAIGASVANPDAIVVDIDGDGSFIMNVQELATIRVENLPVKVLLLNNQHLGMVMQWEDRFYKANRAHTFLGDPAQEDEIFPNMLLFAAACGIPAARVTKKADLREAIQTMLDTPGPYLLDVICPHQEHVLPMIPNGGTFNDVITEGDGRIKY